European Patent Application EP 4 682 167 A1, published January 21, 2026. Title: Therapeutic variable domain of heavy chain (VHH) antibodies against Basigin (CD147) and their use for blocking Plasmodium falciparum entry into human erythrocytes. Applicant: Max-Planck-Gesellschaft zur Foerderung der Wissenschaften e.V. The sequence listing filed with the application follows.

SEQUENCE LISTING (112 sequences)

SEQ ID NO: 1 - protein, 181 aa, Homo sapiens
  source 1..181: note = Basigin Isoform 2 ectodomain (UniProt P35613-2, residues 24-204)
GTVFTTVEDLGSKILLTCSLNDSATEVTGHRWLKGGVVLKEDALPGQKTEFKVDSDDQWGEYSCVFLPEPMGTANIQLHGPPRVKAVKSSEHINEGETAMLVCKSESVPPVTDWAWYKITDSEDKALMNGSESRFFVSSSQGRSELHIENLNMEADPGQYRCNGTSSKGSDQAIITLRVRS

SEQ ID NO: 2 - protein, 192 aa, synthetic construct
  source 1..192: note = Basigin used in BLI experiments
GSECSSGSEPGTVFTTVEDLGSKILLTCSLNDSATEVTGHRWLKGGVVLKEDALPGQKTEFKVDSDDQWGEYSCVFLPEPMGTANIQLHGPPRVKAVKSSEHINEGETAMLVCKSESVPPVTDWAWYKITDSEDKALMNGSESRFFVSSSQGRSELHIENLNMEADPGQYRCNGTSSKGSDQAIITLRVRSC

SEQ ID NO: 3 - protein, 191 aa, synthetic construct
  source 1..191: note = Basigin used in crystallography
GSEGSSGSEPGTVFTTVEDLGSKILLTCSLNDSATEVTGHRWLKGGVVLKEDALPGQKTEFKVDSDDQWGEYSCVFLPEPMGTANIQLHGPPRVKAVKSSEHINEGETAMLVCKSESVPPVTDWAWYKITDSEDKALMNGSESRFFVSSSQGRSELHIENLNMEADPGQYRCNGTSSKGSDQAIITLRVRS

SEQ ID NO: 4 - protein, 502 aa, unidentified
  source 1..502: note = Plasmodium falciparum (isolate 3D7), pfRH5 (UniProt Q8IFM5, residues 25-526; Glycosylation mutant (Crosnier et al., 2013))
FENAIKKTKNQENNLALLPIKSTEEEKDDIKNGKDIKKEIDNDKENIKTNNAKDHSTYIKSYLNTNVNDGLKYLFIPSHNSFIKKYSVFNQINDGMLLNEKNDVKNNEDYKNVDYKNVNFLQYHFKELSNYNIANSIDILQEKEGHLDFVIIPHYTFLDYYKHLSYNSIYHKSSTYGKCIAVDAFIKKINEAYDKVKSKCNDIKNDLIATIKKLEHPYDINNKNDDSYRYDISEEIDDKSEETDDETEEVEDSIQDTDSNHAPSNKKKNDLMNRAFKKMMDEYNTKKKKLIKCIKNHENDFNKICMDMKNYGTNLFEQLSCYNNNFCNTNGIRYHYDEYIHKLILSVKSKNLNKDLSDMTNILQQSELLLTNLNKKMGSYIYIDTIKFIHKEMKHIFNRIEYHTKIINDKTKIIQDKIKLNIWRTFQKDELLKRILDMSNEYSLFITSDHLRQMLYNTFYSKEKHLNNIFHHLIYVLQMKFNDVPIKMEYFQTYKKNKPLTQ

SEQ ID NO: 5 - protein, 125 aa, synthetic construct
  source 1..125: note = Bm7D12
QVQLVESGGGLVQPGGSLRLSCAASGLGSYGVGWFRQAPGKEREGVSCMSTSGRVSYDADSVKGRFTISRDNAKNTSTLQMNSLRPEDSGIYYCAKVRYLAYGDKVCLADEDTIWGLGTLVTVSS

SEQ ID NO: 6 - protein, 11 aa, synthetic construct
  source 1..11: note = Bm7D12_CDR1
GLGSYGVGWFR

SEQ ID NO: 7 - protein, 16 aa, synthetic construct
  source 1..16: note = Bm7D12_CDR2
GVSCMSTSGRVSYDAD

SEQ ID NO: 8 - protein, 21 aa, synthetic construct
  source 1..21: note = Bm7D12_CDR3
AKVRYLAYGDKVCLADEDTIW

SEQ ID NO: 9 - protein, 125 aa, synthetic construct
  source 1..125: note = Bm7H08
QVQLVESGGGWVRPGGSLTLSCTGAGLGNYGIGWFHQAPGKEREGVSCMSTSGRVTYDVDSVKGRFTISRDNAKNTSTLQMNNLRPEDSGIYYCAKVRYLAYGDKVCLADENASWGLGTLVTVSS

SEQ ID NO: 10 - protein, 11 aa, synthetic construct
  source 1..11: note = Bm7H08_CDR1
GLGNYGIGWFH

SEQ ID NO: 11 - protein, 16 aa, synthetic construct
  source 1..16: note = Bm7H08_CDR2
GVSCMSTSGRVTYDVD

SEQ ID NO: 12 - protein, 21 aa, synthetic construct
  source 1..21: note = Bm7H08_CDR3
AKVRYLAYGDKVCLADENASW

SEQ ID NO: 13 - protein, 125 aa, synthetic construct
  source 1..125: note = Bm7G12
QVQLVESGGGWVRPGESLTLSCTGAGLGNYGIGWFHQAPGKEREGVSCMSTSGRVTYDVDSVKGRFTISRDNAKNTSTLQMNNLRPEDSGIYYCAKVRYLAYGDKVCLADENASWGLGTQVTVSS

SEQ ID NO: 14 - protein, 11 aa, synthetic construct
  source 1..11: note = Bm7G12_CDR1
GLGNYGIGWFH

SEQ ID NO: 15 - protein, 16 aa, synthetic construct
  source 1..16: note = Bm7G12_CDR2
GVSCMSTSGRVTYDVD

SEQ ID NO: 16 - protein, 21 aa, synthetic construct
  source 1..21: note = Bm7G12_CDR3
AKVRYLAYGDKVCLADENASW

SEQ ID NO: 17 - protein, 125 aa, synthetic construct
  source 1..125: note = Bm7E11
QVQLVESGGGSVQPGGSLRLSCTGSGLGNYGIGWFRQAPGKEREGVSCMSSSGRVTYNVDSVEGRFTISRDNAKNTSTLEMNSLRPEDSGIYYCAKVRYLAYGDKVCLADENASWGLGTQVTVSS

SEQ ID NO: 18 - protein, 11 aa, synthetic construct
  source 1..11: note = Bm7E11_CDR1
GLGNYGIGWFR

SEQ ID NO: 19 - protein, 16 aa, synthetic construct
  source 1..16: note = Bm7E11_CDR2
GVSCMSSSGRVTYNVD

SEQ ID NO: 20 - protein, 21 aa, synthetic construct
  source 1..21: note = Bm7E11_CDR3
AKVRYLAYGDKVCLADENASW

SEQ ID NO: 21 - protein, 125 aa, synthetic construct
  source 1..125: note = Bm7F03
QVQLVESGGGWVQPGGSLRLSCTGSGLGNYGIGWFRQAPGKEREGVSCMSSSGRVTYNVDSVEGRFTISRDNAKNTSTLEMNSLRPEDSGIYYCAKVRYLAYGDKVCLADENAYWGQGTQVTVSS

SEQ ID NO: 22 - protein, 11 aa, synthetic construct
  source 1..11: note = Bm7F03_CDR1
GLGNYGIGWFR

SEQ ID NO: 23 - protein, 16 aa, synthetic construct
  source 1..16: note = Bm7F03_CDR2
GVSCMSSSGRVTYNVD

SEQ ID NO: 24 - protein, 21 aa, synthetic construct
  source 1..21: note = Bm7F03_CDR3
AKVRYLAYGDKVCLADENAYW

SEQ ID NO: 25 - protein, 125 aa, synthetic construct
  source 1..125: note = Bm7G08
QVQLVESGGGWVRPGGSLTLSCTGAGLGNYGIGWFYQAPGKEREGVSCMSTSGRVTYDVDSVKGRFTISRDNAKNTSTLQMNNLRPEDSGIYYCAKVRYLAYGDKVCLADENASWGLGTQVTVSS

SEQ ID NO: 26 - protein, 11 aa, synthetic construct
  source 1..11: note = Bm7G08_CDR1
GLGNYGIGWFY

SEQ ID NO: 27 - protein, 16 aa, synthetic construct
  source 1..16: note = Bm7G08_CDR2
GVSCMSTSGRVTYDVD

SEQ ID NO: 28 - protein, 21 aa, synthetic construct
  source 1..21: note = Bm7G08_CDR3
AKVRYLAYGDKVCLADENASW

SEQ ID NO: 29 - protein, 125 aa, synthetic construct
  source 1..125: note = Bm27D04
QVQLVESGGGWVRPGESLTLSCTGAGLGKSGIGWFHQAPGKEREGVSCMSTSGRVSYDADSVKGRFTISRDNAKNTSTLQMNSLTPDDSGMYFCARVHYLAYGDRICLADDNASWGPGTQVTVSS

SEQ ID NO: 30 - protein, 11 aa, synthetic construct
  source 1..11: note = Bm27D04_CDR1
GLGKSGIGWFH

SEQ ID NO: 31 - protein, 16 aa, synthetic construct
  source 1..16: note = Bm27D04_CDR2
GVSCMSTSGRVSYDAD

SEQ ID NO: 32 - protein, 21 aa, synthetic construct
  source 1..21: note = Bm27D04_CDR3
ARVHYLAYGDRICLADDNASW

SEQ ID NO: 33 - protein, 125 aa, synthetic construct
  source 1..125: note = Bm27H02
QVQLVESGGGLVKPGGSLTLSCSASGLGSYGIGWFRQAPGKEREGVSCMSTSGRVSYDADSVKGRFTISRDNAKNTSTLQMNNLRPEDSGIYYCAKVRYLAYGDKVCLADEYTSWGLGTQVTVSS

SEQ ID NO: 34 - protein, 11 aa, synthetic construct
  source 1..11: note = Bm27H02_CDR1
GLGSYGIGWFR

SEQ ID NO: 35 - protein, 16 aa, synthetic construct
  source 1..16: note = Bm27H02_CDR2
GVSCMSTSGRVSYDAD

SEQ ID NO: 36 - protein, 21 aa, synthetic construct
  source 1..21: note = Bm27H02_CDR3
AKVRYLAYGDKVCLADEYTSW

SEQ ID NO: 37 - protein, 127 aa, synthetic construct
  source 1..127: note = Bm8D12
QVQLVESGGGLVQAGDSLRLSCAASGRSFSNYAMGWFRQAPGKEREFVSATSWSDGTNYYAEASESVKGRFTTSRDNGNAMTLTMKRLKPEDTAIYYCAARGSTGWATKEAQDYVYWGQGTQVTVSS

SEQ ID NO: 38 - protein, 13 aa, synthetic construct
  source 1..13: note = Bm8D12_CDR1
GRSFSNYAMGWFR

SEQ ID NO: 39 - protein, 19 aa, synthetic construct
  source 1..19: note = Bm8D12_CDR2
FVSATSWSDGTNYYAEASE

SEQ ID NO: 40 - protein, 19 aa, synthetic construct
  source 1..19: note = Bm8D12_CDR3
AARGSTGWATKEAQDYVYW

SEQ ID NO: 41 - protein, 127 aa, synthetic construct
  source 1..127: note = Bm8B10
QVQLVESGGGLVQAGDSLRLSCAGSGRTFTNVAMAWFRQASGKEREFVSGISWTGGTSYYAEADDSVKGRFTLSRDNANMVTLKMNSLKPEDTAVYYCAARESAGWATKKAQDYVYWGQGTQVTVSS

SEQ ID NO: 42 - protein, 13 aa, synthetic construct
  source 1..13: note = Bm8B10_CDR1
GRTFTNVAMAWFR

SEQ ID NO: 43 - protein, 19 aa, synthetic construct
  source 1..19: note = Bm8B10_CDR2
FVSGISWTGGTSYYAEADD

SEQ ID NO: 44 - protein, 19 aa, synthetic construct
  source 1..19: note = Bm8B10_CDR3
AARESAGWATKKAQDYVYW

SEQ ID NO: 45 - protein, 127 aa, synthetic construct
  source 1..127: note = Bm8D09
QVQLVESGGGQVQAGDSLSLSCAASGRTFTNYAMAWFRQASGKEREFVSGISWTGGTSYYAEADDSVKGRFTLSRDNANMVTLKMNRLKPEDTAVYYCAARESAGWATKKAQDYVYWGQGTQVTVSS

SEQ ID NO: 46 - protein, 13 aa, synthetic construct
  source 1..13: note = Bm8D09_CDR1
GRTFTNYAMAWFR

SEQ ID NO: 47 - protein, 19 aa, synthetic construct
  source 1..19: note = Bm8D09_CDR2
FVSGISWTGGTSYYAEADD

SEQ ID NO: 48 - protein, 19 aa, synthetic construct
  source 1..19: note = Bm8D09_CDR3
AARESAGWATKKAQDYVYW

SEQ ID NO: 49 - protein, 127 aa, synthetic construct
  source 1..127: note = Bm8H12
QVQLVESGGGLVQAGDSLTLSCTASGRTFENYAMGWFRQAPGKEREFVSATSWTGGTNYYAEASESVKGRFTTSRDNGNKVTLKMNRLKPEDTAIYYCAVRGSTGWATKRAQEYDYWGQGTQVTVSS

SEQ ID NO: 50 - protein, 13 aa, synthetic construct
  source 1..13: note = Bm8H12_CDR1
GRTFENYAMGWFR

SEQ ID NO: 51 - protein, 19 aa, synthetic construct
  source 1..19: note = Bm8H12_CDR2
FVSATSWTGGTNYYAEASE

SEQ ID NO: 52 - protein, 19 aa, synthetic construct
  source 1..19: note = Bm8H12_CDR3
AVRGSTGWATKRAQEYDYW

SEQ ID NO: 53 - protein, 127 aa, synthetic construct
  source 1..127: note = Bm8C06
QVQLVESGGGLVQAGSSLRLSCAASGRTFTNYAMGWFRQAPGKEREFVSATSWTGDTNYYAEATESVKGRFTTSRDNDNTVTLQMKRLKPEDTGIYYCAARGSAGWATQQAQDYVYWGQGTQVTVSS

SEQ ID NO: 54 - protein, 13 aa, synthetic construct
  source 1..13: note = Bm8C06_CDR1
GRTFTNYAMGWFR

SEQ ID NO: 55 - protein, 19 aa, synthetic construct
  source 1..19: note = Bm8C06_CDR2
FVSATSWTGDTNYYAEATE

SEQ ID NO: 56 - protein, 19 aa, synthetic construct
  source 1..19: note = Bm8C06_CDR3
AARGSAGWATQQAQDYVYW

SEQ ID NO: 57 - protein, 127 aa, synthetic construct
  source 1..127: note = Bm8H07
QVQLVESGGGTVQIGDSLTLSCESSEGLFSNYAMGWFRQAPGKEREFVSATSWNGGTNYYAEAAESVKGRFTTSRDNANKVTLKMNRLKPEDTAIYYCAARDSEGWATKNAQEYVYWGQGTQVTVSS

SEQ ID NO: 58 - protein, 13 aa, synthetic construct
  source 1..13: note = Bm8H07_CDR1
EGLFSNYAMGWFR

SEQ ID NO: 59 - protein, 19 aa, synthetic construct
  source 1..19: note = Bm8H07_CDR2
FVSATSWNGGTNYYAEAAE

SEQ ID NO: 60 - protein, 19 aa, synthetic construct
  source 1..19: note = Bm8H07_CDR3
AARDSEGWATKNAQEYVYW

SEQ ID NO: 61 - protein, 127 aa, synthetic construct
  source 1..127: note = Bm8G09
QVQLVESGGGLVQAGDSLTLSCTASGRTFENYAMGWFRQAPGKEREFVSAISWTGGTNYVAETTESLRGRFTLSRDNANMVTLKTNRLEPEDTAIYYCAARGSTGWATKEAQDYVYWGQGTQVTVSS

SEQ ID NO: 62 - protein, 13 aa, synthetic construct
  source 1..13: note = Bm8G09_CDR1
GRTFENYAMGWFR

SEQ ID NO: 63 - protein, 19 aa, synthetic construct
  source 1..19: note = Bm8G09_CDR2
FVSAISWTGGTNYVAETTE

SEQ ID NO: 64 - protein, 19 aa, synthetic construct
  source 1..19: note = Bm8G09_CDR3
AARGSTGWATKEAQDYVYW

SEQ ID NO: 65 - protein, 118 aa, synthetic construct
  source 1..118: note = Bm8G10
QVQLVESGGGLVQSGGSLRLSCAASGFTLDAYAIGWFRQAPGKERERVSCIGSGGGAALYADSVKGRFTVSRDNAKNTVYLQMNSLKPEDTALYFCAGDCSASAYSLKGQGTQVTVSS

SEQ ID NO: 66 - protein, 13 aa, synthetic construct
  source 1..13: note = Bm8G10_CDR1
GFTLDAYAIGWFR

SEQ ID NO: 67 - protein, 16 aa, synthetic construct
  source 1..16: note = Bm8G10_CDR2
RVSCIGSGGGAALYAD

SEQ ID NO: 68 - protein, 12 aa, synthetic construct
  source 1..12: note = Bm8G10_CDR3
AGDCSASAYSLK

SEQ ID NO: 69 - protein, 118 aa, synthetic construct
  source 1..118: note = Bm8F05
QVQLVESGGGLVQPGGSLRLSCQASGITLNQYAIGWFRQAPGKEREVLSCIGSGAGGTRYADSVKGRFTISRDNAKSTVYLQMNSLKLEDTALYYCAADCSGGPYSLRGQGTQVTVSS

SEQ ID NO: 70 - protein, 13 aa, synthetic construct
  source 1..13: note = Bm8F05_CDR1
GITLNQYAIGWFR

SEQ ID NO: 71 - protein, 16 aa, synthetic construct
  source 1..16: note = Bm8F05_CDR2
VLSCIGSGAGGTRYAD

SEQ ID NO: 72 - protein, 12 aa, synthetic construct
  source 1..12: note = Bm8F05_CDR3
AADCSGGPYSLR

SEQ ID NO: 73 - protein, 124 aa, synthetic construct
  source 1..124: note = Bm8H10
QVQLVESGGGFVQPGGSLRLSCAAPGSTLDGYSIGWFRQAPGKEREGVGCISRSSANRSYKDYVKGRFTISRDKNTVYLEMKSLKPEDTAVYICAAQETEDQHACYYYRGMDYWGKGTQVTVSS

SEQ ID NO: 74 - protein, 13 aa, synthetic construct
  source 1..13: note = Bm8H10_CDR1
GSTLDGYSIGWFR

SEQ ID NO: 75 - protein, 16 aa, synthetic construct
  source 1..16: note = Bm8H10_CDR2
GVGCISRSSANRSYKD

SEQ ID NO: 76 - protein, 20 aa, synthetic construct
  source 1..20: note = Bm8H10_CDR3
AAQETEDQHACYYYRGMDYW

SEQ ID NO: 77 - protein, 127 aa, synthetic construct
  source 1..127: note = Bm8G06
QVQLVESGGGLVQPGGSLRLSCSGSGSTLDHFSIGWFRQTPGKEREGVGCISWSGRNRAYKDYVKGRFTISRDDAKNTVYLEMNFLKPEDTGVYYCAAQEAVDWPDACYYYAGMPYWGKGTQVTVSS

SEQ ID NO: 78 - protein, 13 aa, synthetic construct
  source 1..13: note = Bm8G06_CDR1
GSTLDHFSIGWFR

SEQ ID NO: 79 - protein, 16 aa, synthetic construct
  source 1..16: note = Bm8G06_CDR2
GVGCISWSGRNRAYKD

SEQ ID NO: 80 - protein, 21 aa, synthetic construct
  source 1..21: note = Bm8G06_CDR3
AAQEAVDWPDACYYYAGMPYW

SEQ ID NO: 81 - protein, 128 aa, synthetic construct
  source 1..128: note = Bm8G07
QVQLVESGGTLVQPGGSLRLSCQASGFTLGRYPIGWYRQAPGKEREGVACITGDGDLVDYNYRMEGRFTISRDNARNTVYLQMNSLDPEDTAIYYCAAQVSSRSLCSLLKPFGGMEYWGEGTLVTVSS

SEQ ID NO: 82 - protein, 13 aa, synthetic construct
  source 1..13: note = Bm8G07_CDR1
GFTLGRYPIGWYR

SEQ ID NO: 83 - protein, 16 aa, synthetic construct
  source 1..16: note = Bm8G07_CDR2
GVACITGDGDLVDYNY

SEQ ID NO: 84 - protein, 22 aa, synthetic construct
  source 1..22: note = Bm8G07_CDR3
AAQVSSRSLCSLLKPFGGMEYW

SEQ ID NO: 85 - protein, 111 aa, synthetic construct
  source 1..111: note = Bm8G12
QVQLVESGGGLVQAGDSLRLSCAASEGIFVNHGMGWYRQVPGNEREWVAIMFGTGGTKYQDSVKGRFTISRDNAKNTVDLQMNSLKPEDTGIYYCNQGSIWGQGTQVTVSS

SEQ ID NO: 86 - protein, 13 aa, synthetic construct
  source 1..13: note = Bm8G12_CDR1
EGIFVNHGMGWYR

SEQ ID NO: 87 - protein, 15 aa, synthetic construct
  source 1..15: note = Bm8G12_CDR2
WVAIMFGTGGTKYQD

SEQ ID NO: 88 - protein, 6 aa, synthetic construct
  source 1..6: note = Bm8G12_CDR3
NQGSIW

SEQ ID NO: 89 - protein, 111 aa, synthetic construct
  source 1..111: note = Bm27C04
QVQLVESGGGLVQPGGSLRLSCGASEGIFVNHGMGWYHQVPGHEREWVAIMFGTGGTKYQDSVKGRFTISRDNAKNTVDLQMNSLKPEDTGIYYCNQGSIWGQGTQVTVSS

SEQ ID NO: 90 - protein, 13 aa, synthetic construct
  source 1..13: note = Bm27C04_CDR1
EGIFVNHGMGWYH

SEQ ID NO: 91 - protein, 15 aa, synthetic construct
  source 1..15: note = Bm27C04_CDR2
WVAIMFGTGGTKYQD

SEQ ID NO: 92 - protein, 6 aa, synthetic construct
  source 1..6: note = Bm27C04_CDR3
NQGSIW

SEQ ID NO: 93 - protein, 111 aa, synthetic construct
  source 1..111: note = Bm27C06
QVQLVESGGGLVQTGGSLRLSCAASEGIRVNHGMGWYRQVPGNEREWVAIMFGTGGTKYQDSVKGRFTISRDNAKNTVDLQMNSLKPEDTGIYYCNQGSIWGQGTQVTVSS

SEQ ID NO: 94 - protein, 13 aa, synthetic construct
  source 1..13: note = Bm27C06_CDR1
EGIRVNHGMGWYR

SEQ ID NO: 95 - protein, 15 aa, synthetic construct
  source 1..15: note = Bm27C06_CDR2
WVAIMFGTGGTKYQD

SEQ ID NO: 96 - protein, 6 aa, synthetic construct
  source 1..6: note = Bm27C06_CDR3
NQGSIW

SEQ ID NO: 97 - protein, 118 aa, synthetic construct
  source 1..118: note = Bm27E06
QVQLVESGGGTVQPGGSLRLSCAASRLTVDQYAIGWFRQAPGKEQERVSCIGAGGGAAIYADSVKGRFTVSRDNAKNTVYLQMNSLKPEDTAVYFCAGDCSASAYSLKGQGTLVTVSS

SEQ ID NO: 98 - protein, 13 aa, synthetic construct
  source 1..13: note = Bm27E06_CDR1
RLTVDQYAIGWFR

SEQ ID NO: 99 - protein, 16 aa, synthetic construct
  source 1..16: note = Bm27E06_CDR2
RVSCIGAGGGAAIYAD

SEQ ID NO: 100 - protein, 12 aa, synthetic construct
  source 1..12: note = Bm27E06_CDR3
AGDCSASAYSLK

SEQ ID NO: 101 - protein, 118 aa, synthetic construct
  source 1..118: note = Bm27H03
QVQLVESGGGTVQPGGSLRLSCAASGLTVDAYAIGWFRQAPGKERERVSCIGSGGGAAIYADSVKGRFTVSRGNAKNTVYLQMNSLKPEDTGVYFCAGDCSASAYSLKGQGTQVTVSS

SEQ ID NO: 102 - protein, 13 aa, synthetic construct
  source 1..13: note = Bm27H03_CDR1
GLTVDAYAIGWFR

SEQ ID NO: 103 - protein, 16 aa, synthetic construct
  source 1..16: note = Bm27H03_CDR2
RVSCIGSGGGAAIYAD

SEQ ID NO: 104 - protein, 12 aa, synthetic construct
  source 1..12: note = Bm27H03_CDR3
AGDCSASAYSLK

SEQ ID NO: 105 - protein, 131 aa, synthetic construct
  source 1..131: note = Bm27C11
QVQLVESGGGLAQPGGSLRLSCAASGFTFSKHAMGWYRQAPGNECELVATISNGGSRTNYADSVKGRFTISRDNAGSTLYLQMNSLKPEDTAVYYCNTGWGAGTEQTACTMSEKFGALDAWGQGTLVTVSS

SEQ ID NO: 106 - protein, 13 aa, synthetic construct
  source 1..13: note = Bm27C11_CDR1
GFTFSKHAMGWYR

SEQ ID NO: 107 - protein, 16 aa, synthetic construct
  source 1..16: note = Bm27C11_CDR2
LVATISNGGSRTNYAD

SEQ ID NO: 108 - protein, 25 aa, synthetic construct
  source 1..25: note = Bm27C11_CDR3
NTGWGAGTEQTACTMSEKFGALDAW

SEQ ID NO: 109 - protein, 131 aa, synthetic construct
  source 1..131: note = Bm27D06
QVQLVESGGGLAQPGGSLRLSCAASGFTFSKHAMGWYRQAPGNECELVATISNGGSRTNYADSVKGRFTISRDNAGSTLYLQMNSLKPEDTAVYYCNTGWGAGTEQTACTMSEKFGALDAWGQGTQVTVSS

SEQ ID NO: 110 - protein, 13 aa, synthetic construct
  source 1..13: note = Bm27D06_CDR1
GFTFSKHAMGWYR

SEQ ID NO: 111 - protein, 16 aa, synthetic construct
  source 1..16: note = Bm27D06_CDR2
LVATISNGGSRTNYAD

SEQ ID NO: 112 - protein, 25 aa, synthetic construct
  source 1..25: note = Bm27D06_CDR3
NTGWGAGTEQTACTMSEKFGALDAW